European Patent Application EP 4 613 853 A1, published September 10, 2025. Title: Mutant microorganism of Corynebacterium genus producing L-glutamic acid and method for producing L-glutamic acid using the same. Applicant: DAESANG CORPORATION. The sequence listing filed with the application follows.

SEQUENCE LISTING (9 sequences)

SEQ ID NO: 1 - DNA, 801 bp, synthetic construct
  source 1..801: mol_type = other DNA
ttgagtttcacgcatggtcagggcagagtttttgataccgtcgagcagatccgcatgttcggcagcgccctgcgcaaaaccggcaaaccagtggtgctcgtacacttgggaaatggcctccacgcaggccatattgcgctcatccgcgcagcaaaacgcatccccggtgcggtggtcgtcgtcgcctatgccggcccggaatcggatcacgcacgtttaagggaagagcttatcgacgcgatcttcccgttcaatcccgaaacgctatggcctcacggcatccgggtggaagttacaggtggcccaacacttaccccacaaggtgcggaagtaaccaaggtgctgggtctgttgggaatcaccggagcaactgatgtggtgctcggtgaaaaggattatgaactggtggttctagtccagcgcgcactcaacgatctgcatattccagtaaaactgcattctgttccaaccgtgcgcatgccagacggccttgctatttctctgcgtaacgtttcagtgtccgaagactcccgtgaaaccgcattgagcctggcagcagccctcaccgccggtgcacactccgcagaacacggcgaagcagtggttaaagaaacagtcacgcaagtactcaaagccgccggcgtgacccccgattatgtagaaatccgtggcctggatcttggactagcccccgaaatcggagacgcccgactcttcgcagccatcacccttggagatgtccaactccacgacaacgtcggcctaccgcttggaatcggcttcaaaaacatcgaaggctga

SEQ ID NO: 2 - protein, 266 aa, synthetic construct
LSFTHGQGRVFDTVEQIRMFGSALRKTGKPVVLVHLGNGLHAGHIALIRAAKRIPGAVVVVAYAGPESDHARLREELIDAIFPFNPETLWPHGIRVEVTGGPTLTPQGAEVTKVLGLLGITGATDVVLGEKDYELVVLVQRALNDLHIPVKLHSVPTVRMPDGLAISLRNVSVSEDSRETALSLAAALTAGAHSAEHGEAVVKETVTQVLKAAGVTPDYVEIRGLDLGLAPEIGDARLFAAITLGDVQLHDNVGLPLGIGFKNIEG

SEQ ID NO: 3 - DNA, 801 bp, Corynebacterium sp.
  source 1..801: mol_type = genomic DNA
ttgagtttcacgcatggtcagggcagagtttttgataccgtcgagcagatccgcatgttcggcagcgccctgcgcaaaaccggcaaaccagtggtgctcgtacacttgggaaatggcctccacgcaggccatattgcgctcatccgcgcagcaaaacgcatccccggtgcggtggtcgtcgtcgcctatgccggcccggaatcggatcacgcacgtttaagggaagagcttatcgacgcgatcttcccgttcaatcccgaaacgctatggcctcacggcatccgggtggaagttacaggtggcccaacacttaccccacaaggtgcggaagtaaccaaggtgctgggtctgttgggaatcaccggagcaactgatgtggtgctcggtgaaaaggattatgaactggtggttctagtccagcgcgcactcaacgatctgcatattccagtaaaactgcattctgttccaaccgtgcgcatgccagacggccttgctatttctctgcgtaacgtttcagtgcccgaagactcccgtgaaaccgcattgagcctggcagcagccctcaccgccggtgcacactccgcagaacacggcgaagcagtggttaaagaaacagtcacgcaagtactcaaagccgccggcgtgacccccgattatgtagaaatccgtggcctggatcttggactagcccccgaaatcggagacgcccgactcttcgcagccatcacccttggagatgtccaactccacgacaacgtcggcctaccgcttggaatcggcttcaaaaacatcgaaggctga

SEQ ID NO: 4 - protein, 266 aa, Corynebacterium sp.
LSFTHGQGRVFDTVEQIRMFGSALRKTGKPVVLVHLGNGLHAGHIALIRAAKRIPGAVVVVAYAGPESDHARLREELIDAIFPFNPETLWPHGIRVEVTGGPTLTPQGAEVTKVLGLLGITGATDVVLGEKDYELVVLVQRALNDLHIPVKLHSVPTVRMPDGLAISLRNVSVPEDSRETALSLAAALTAGAHSAEHGEAVVKETVTQVLKAAGVTPDYVEIRGLDLGLAPEIGDARLFAAITLGDVQLHDNVGLPLGIGFKNIEG

SEQ ID NO: 5 - DNA, 5719 bp, synthetic construct
  source 1..5719: mol_type = other DNA
tgccgcaagcactcagggcgcaagggctgctaaaggaagcggaacacgtagaaagccagtccgcagaaacggtgctgaccccggatgaatgtcagctactgggctatctggacaagggaaaacgcaagcgcaaagagaaagcaggtagcttgcagtgggcttacatggcgatagctagactgggcggttttatggacagcaagcgaaccggaattgccagctggggcgccctctggtaaggttgggaagccctgcaaagtaaactggatggctttcttgccgccaaggatctgatggcgcaggggatcaagatctgatcaagagacaggatgaggatcgtttcgcatgattgaacaagatggattgcacgcaggttctccggccgcttgggtggagaggctattcggctatgactgggcacaacagacaatcggctgctctgatgccgccgtgttccggctgtcagcgcaggggcgcccggttctttttgtcaagaccgacctgtccggtgccctgaatgaactccaagacgaggcagcgcggctatcgtggctggccacgacgggcgttccttgcgcagctgtgctcgacgttgtcactgaagcgggaagggactggctgctattgggcgaagtgccggggcaggatctcctgtcatctcaccttgctcctgccgagaaagtatccatcatggctgatgcaatgcggcggctgcatacgcttgatccggctacctgcccattcgaccaccaagcgaaacatcgcatcgagcgagcacgtactcggatggaagccggtcttgtcgatcaggatgatctggacgaagagcatcaggggctcgcgccagccgaactgttcgccaggctcaaggcgcggatgcccgacggcgaggatctcgtcgtgacccatggcgatgcctgcttgccgaatatcatggtggaaaatggccgcttttctggattcatcgactgtggccggctgggtgtggcggaccgctatcaggacatagcgttggctacccgtgatattgctgaagagcttggcggcgaatgggctgaccgcttcctcgtgctttacggtatcgccgctcccgattcgcagcgcatcgccttctatcgccttcttgacgagttcttctgagcgggactctggggttcgctagaggatcgatcctttttaacccatcacatatacctgccgttcactattatttagtgaaatgagatattatgatattttctgaattgtgattaaaaaggcaactttatgcccatgcaacagaaactataaaaaatacagagaatgaaaagaaacagatagattttttagttctttaggcccgtagtctgcaaatccttttatgattttctatcaaacaaaagaggaaaatagaccagttgcaatccaaacgagagtctaatagaatgaggtcgaaaagtaaatcgcgcgggtttgttactgataaagcaggcaagacctaaaatgtgtaaagggcaaagtgtatactttggcgtcaccccttacatattttaggtctttttttattgtgcgtaactaacttgccatcttcaaacaggagggctggaagaagcagaccgctaacacagtacataaaaaaggagacatgaacgatgaacatcaaaaagtttgcaaaacaagcaacagtattaacctttactaccgcactgctggcaggaggcgcaactcaagcgtttgcgaaagaaacgaaccaaaagccatataaggaaacatacggcatttcccatattacacgccatgatatgctgcaaatccctgaacagcaaaaaaatgaaaaatatcaagtttctgaatttgattcgtccacaattaaaaatatctcttctgcaaaaggcctggacgtttgggacagctggccattacaaaacgctgacggcactgtcgcaaactatcacggctaccacatcgtctttgcattagccggagatcctaaaaatgcggatgacacatcgatttacatgttctatcaaaaagtcggcgaaacttctattgacagctggaaaaacgctggccgcgtctttaaagacagcgacaaattcgatgcaaatgattctatcctaaaagaccaaacacaagaatggtcaggttcagccacatttacatctgacggaaaaatccgtttattctacactgatttctccggtaaacattacggcaaacaaacactgacaactgcacaagttaacgtatcagcatcagacagctctttgaacatcaacggtgtagaggattataaatcaatctttgacggtgacggaaaaacgtatcaaaatgtacagcagttcatcgatgaaggcaactacagctcaggcgacaaccatacgctgagagatcctcactacgtagaagataaaggccacaaatacttagtatttgaagcaaacactggaactgaagatggctaccaaggcgaagaatctttatttaacaaagcatactatggcaaaagcacatcattcttccgtcaagaaagtcaaaaacttctgcaaagcgataaaaaacgcacggctgagttagcaaacggcgctctcggtatgattgagctaaacgatgattacacactgaaaaaagtgatgaaaccgctgattgcatctaacacagtaacagatgaaattgaacgcgcgaacgtctttaaaatgaacggcaaatggtacctgttcactgactcccgcggatcaaaaatgacgattgacggcattacgtctaacgatatttacatgcttggttatgtttctaattctttaactggcccatacaagccgctgaacaaaactggccttgtgttaaaaatggatcttgatcctaacgatgtaacctttacttactcacacttcgctgtacctcaagcgaaaggaaacaatgtcgtgattacaagctatatgacaaacagaggattctacgcagacaaacaatcaacgtttgcgccgagcttcctgctgaacatcaaaggcaagaaaacatctgttgtcaaagacagcatccttgaacaaggacaattaacagttaacaaataaaaacgcaaaagaaaatgccgatgggtaccgagcgaaatgaccgaccaagcgacgcccaacctgccatcacgagatttcgattccaccgccgccttctatgaaaggttgggcttcggaatcgttttccgggacgccctcgcggacgtgctcatagtccacgacgcccgtgattttgtagccctggccgacggccagcaggtaggccgacaggctcatgccggccgccgccgccttttcctcaatcgctcttcgttcgtctggaaggcagtacaccttgataggtgggctgcccttcctggttggcttggtttcatcagccatccgcttgccctcatctgttacgccggcggtagccggccagcctcgcagagcaggattcccgttgagcaccgccaggtgcgaataagggacagtgaagaaggaacacccgctcgcgggtgggcctacttcacctatcctgcccggctgacgccgttggatacaccaaggaaagtctacacgaaccctttggcaaaatcctgtatatcgtgcgaaaaaggatggatataccgaaaaaatcgctataatgaccccgaagcagggttatgcagcggaaaagcgctgcttccctgctgttttgtggaatatctaccgactggaaacaggcaaatgcaggaaattactgaactgaggggacaggcgagagacgatgccaaagagctcctgaaaatctcgataactcaaaaaatacgcccggtagtgatcttatttcattatggtgaaagttggaacctcttacgtgccgatcaacgtctcattttcgccaaaagttggcccagggcttcccggtatcaacagggacaccaggatttatttattctgcgaagtgatcttccgtcacaggtatttattcggcgcaaagtgcgtcgggtgatgctgccaacttactgatttagtgtatgatggtgtttttgaggtgctccagtggcttctgtttctatcagctcctgaaaatctcgataactcaaaaaatacgcccggtagtgatcttatttcattatggtgaaagttggaacctcttacgtgccgatcaacgtctcattttcgccaaaagttggcccagggcttcccggtatcaacagggacaccaggatttatttattctgcgaagtgatcttccgtcacaggtatttattcggcgcaaagtgcgtcgggtgatgctgccaacttactgatttagtgtatgatggtgtttttgaggtgctccagtggcttctgtttctatcagggctggatgatcctccagcgcggggatctcatgctggagttcttcgcccaccccaaaaggatctaggtgaagatcctttttgataatctcatgaccaaaatcccttaacgtgagttttcgttccactgagcgtcagaccccgtagaaaagatcaaaggatcttcttgagatcctttttttctgcgcgtaatctgctgcttgcaaacaaaaaaaccaccgctaccagcggtggtttgtttgccggatcaagagctaccaactctttttccgaaggtaactggcttcagcagagcgcagataccaaatactgttcttctagtgtagccgtagttaggccaccacttcaagaactctgtagcaccgcctacatacctcgctctgctaatcctgttaccagtggctgctgccagtggcgataagtcgtgtcttaccgggttggactcaagacgatagttaccggataaggcgcagcggtcgggctgaacggggggttcgtgcacacagcccagcttggagcgaacgacctacaccgaactgagatacctacagcgtgagctatgagaaagcgccacgcttcccgaagggagaaaggcggacaggtatccggtaagcggcagggtcggaacaggagagcgcacgagggagcttccagggggaaacgcctggtatctttatagtcctgtcgggtttcgccacctctgacttgagcgtcgatttttgtgatgctcgtcaggggggcggagcctatggaaaaacgccagcaacgcggcctttttacggttcctggccttttgctggccttttgctcacatgttctttcctgcgttatcccctgattctgtggataaccgtattaccgcctttgagtgagctgataccgctcgccgcagccgaacgaccgagcgcagcgagtcagtgagcgaggaagcggaagagcgcccaatacgcaaaccgcctctccccgcgcgttggccgattcattaatgcagctggcacgacaggtttcccgactggaaagcgggcagtgagcgcaacgcaattaatgtgagttagctcactcattaggcaccccaggctttacactttatgcttccggctcgtatgttgtgtggaattgtgagcggataacaatttcacacaggaaacagctatgacatgattacgccaagcttgcatgcctgcaggtcgactctagaggatccccgggtaccgagctcgaattcactggccgtcgttttacaacgtcgtgactgggaaaaccctggcgttacccaacttaatcgccttgcagcacatccccctttcgccagctggcgtaatagcgaagaggcccgcaccgatcgcccttcccaacagttgcgcagcctgaatggcgaatggcgataagctagcttcacgc

SEQ ID NO: 6 - DNA, 21 bp, synthetic construct
  source 1..21: mol_type = other DNA
ggtgatcccgatgtgacctct

SEQ ID NO: 7 - DNA, 22 bp, synthetic construct
  source 1..22: mol_type = other DNA
ggagtcttcggacactgaaacg

SEQ ID NO: 8 - DNA, 22 bp, synthetic construct
  source 1..22: mol_type = other DNA
cgtttcagtgtccgaagactcc

SEQ ID NO: 9 - DNA, 20 bp, synthetic construct
  source 1..20: mol_type = other DNA
cttcgctgaggtccgcgaat